European Patent Application EP 4 253 408 A1, published October 4, 2023. Title: TCR CAPABLE OF RECOGNIZING HPV ANTIGEN. Applicant: XLIFESC, LTD. The sequence listing filed with the application follows.

SEQUENCE LISTING (25 sequences)

SEQ ID NO: 1 - protein, 113 aa, Artificial Sequence
  alpha chain variable domain of TCR
AQKVTQAQTEISVVEKEDVTLDCVYETRDTTYYLFWYKQPPSGELVFLIRRNSFDEQNEISGRYSWNFQKSTSSFNFTITASQVVDSAVYFCALRAGANNLFFGTGTRLTVIP

SEQ ID NO: 2 - protein, 113 aa, Artificial Sequence
  alpha chain variable domain of TCR
AQKVTQAQTEISVVEKEDVTLDCVYETRDTTYYLFWYKQPPSGELVFLIRRNSFDEQNEISGRYSWNFQKSTSSFNFTITASQVVDSAVYFCALRAGANLPVFGTGTRLTVIP

SEQ ID NO: 3 - protein, 113 aa, Artificial Sequence
  alpha chain variable domain of TCR
AQKVTQAQTEISVVEKEDVTLDCVYETRDTTYYLFWYKQPPSGELVFLIRRNSFDEQNEISGRYSWNFQKSTSSFNFTITASQVVDSAVYFCALRAGANTPIFGTGTRLTVIP

SEQ ID NO: 4 - protein, 113 aa, Artificial Sequence
  alpha chain variable domain of TCR
AQKVTQAQTEISVVEKEDVTLDCVYETRDTTYYLFWYKQPPSGELVFLIRRNSFDEQNEISGRYSWNFQKSTSSFNFTITASQVVDSAVYFCALRAGAWPMKFGTGTRLTVIP

SEQ ID NO: 5 - protein, 114 aa, Artificial Sequence
  beta chain variable domain of TCR
NAGVTQTPKFQVLKTGQSMTLQCAQDMNHNSMYWYRQDPGMGLRLIYYSASEGTTDKGEVPNGYNVSRLNKREFSLRLESAAPSQTSVYFCASGPWGSSGNTIYFGEGSWLTVV

SEQ ID NO: 6 - protein, 251 aa, Artificial Sequence
  single stranded TCR
AQKVTQAQTELSVPEGEDVTIDCVYETRDTTYYLFWYKQPPSGELVFLIRRNSFDEQNEISGRYSWNFQKSTSSFNFTITAVQPNDSAVYFCALRAGANNLFFGTGTRLTVTPGGGSEGGGSEGGGSEGGGSEGGTGNAGVTQTPKYLSVKTGQSVTLQCAQDMNHNSMYWYRQDPGQGLRLIYYSASEGTTDKGEIPNRYNVSRLNKREFSLKIESVTPSDTSVYFCASGPWGSSGNTIYFGEGSRLTVD

SEQ ID NO: 7 - protein, 251 aa, Artificial Sequence
  single stranded TCR
AQKVTQAQTELSVPEGEDVTIDCVYETRDTTYYLFWYKQPPSGELVFLIRRNSFDEQNEISGRYSWNFQKSTSSFNFTITAVQPNDSAVYFCALRAGANLPVFGTGTRLTVTPGGGSEGGGSEGGGSEGGGSEGGTGNAGVTQTPKYLSVKTGQSVTLQCAQDMNHNSMYWYRQDPGQGLRLIYYSASEGTTDKGEIPNRYNVSRLNKREFSLKIESVTPSDTSVYFCASGPWGSSGNTIYFGEGSRLTVD

SEQ ID NO: 8 - protein, 251 aa, Artificial Sequence
  single stranded TCR
AQKVTQAQTELSVPEGEDVTIDCVYETRDTTYYLFWYKQPPSGELVFLIRRNSFDEQNEISGRYSWNFQKSTSSFNFTITAVQPNDSAVYFCALRAGANTPIFGTGTRLTVTPGGGSEGGGSEGGGSEGGGSEGGTGNAGVTQTPKYLSVKTGQSVTLQCAQDMNHNSMYWYRQDPGQGLRLIYYSASEGTTDKGEIPNRYNVSRLNKREFSLKIESVTPSDTSVYFCASGPWGSSGNTIYFGEGSRLTVD

SEQ ID NO: 9 - protein, 251 aa, Artificial Sequence
  single stranded TCR
AQKVTQAQTELSVPEGEDVTIDCVYETRDTTYYLFWYKQPPSGELVFLIRRNSFDEQNEISGRYSWNFQKSTSSFNFTITAVQPNDSAVYFCALRAGAWPMKFGTGTRLTVTPGGGSEGGGSEGGGSEGGGSEGGTGNAGVTQTPKYLSVKTGQSVTLQCAQDMNHNSMYWYRQDPGQGLRLIYYSASEGTTDKGEIPNRYNVSRLNKREFSLKIESVTPSDTSVYFCASGPWGSSGNTIYFGEGSRLTVD

SEQ ID NO: 10 - protein, 208 aa, Artificial Sequence
  alpha chain variable domain of soluble TCR
MAQKVTQAQTEISVVEKEDVTLDCVYETRDTTYYLFWYKQPPSGELVFLIRRNSFDEQNEISGRYSWNFQKSTSSFNFTITASQVVDSAVYFCALRAGANNLFFGTGTRLTVIPYIQNPDPAVYQLRDSKSSDKSVCLFTDFDSQTNVSQSKDSDVYITDKTVLDMRSMDFKSNSAVAWSNKSDFACANAFNNSIIPEDTFFCSPESS

SEQ ID NO: 11 - protein, 208 aa, Artificial Sequence
  alpha chain variable domain of soluble TCR
MAQKVTQAQTEISVVEKEDVTLDCVYETRDTTYYLFWYKQPPSGELVFLIRRNSFDEQNEISGRYSWNFQKSTSSFNFTITASQVVDSAVYFCALRAGANLPVFGTGTRLTVIPYIQNPDPAVYQLRDSKSSDKSVCLFTDFDSQTNVSQSKDSDVYITDKTVLDMRSMDFKSNSAVAWSNKSDFACANAFNNSIIPEDTFFCSPESS

SEQ ID NO: 12 - protein, 208 aa, Artificial Sequence
  alpha chain variable domain of soluble TCR
MAQKVTQAQTEISVVEKEDVTLDCVYETRDTTYYLFWYKQPPSGELVFLIRRNSFDEQNEISGRYSWNFQKSTSSFNFTITASQVVDSAVYFCALRAGANTPIFGTGTRLTVIPYIQNPDPAVYQLRDSKSSDKSVCLFTDFDSQTNVSQSKDSDVYITDKTVLDMRSMDFKSNSAVAWSNKSDFACANAFNNSIIPEDTFFCSPESS

SEQ ID NO: 13 - protein, 208 aa, Artificial Sequence
  alpha chain variable domain of soluble TCR
MAQKVTQAQTEISVVEKEDVTLDCVYETRDTTYYLFWYKQPPSGELVFLIRRNSFDEQNEISGRYSWNFQKSTSSFNFTITASQVVDSAVYFCALRAGAWPMKFGTGTRLTVIPYIQNPDPAVYQLRDSKSSDKSVCLFTDFDSQTNVSQSKDSDVYITDKTVLDMRSMDFKSNSAVAWSNKSDFACANAFNNSIIPEDTFFCSPESS

SEQ ID NO: 14 - protein, 245 aa, Artificial Sequence
  beta chain variable domain of soluble TCR
MNAGVTQTPKFQVLKTGQSMTLQCAQDMNHNSMYWYRQDPGMGLRLIYYSASEGTTDKGEVPNGYNVSRLNKREFSLRLESAAPSQTSVYFCASGPWGSSGNTIYFGEGSWLTVVEDLKNVFPPEVAVFEPSECEISHTQKATLVCLATGFYPDHVELSWWVNGKEVHSGVSTDPQPLKEQPALNDSRYALSSRLRVSATFWQNPRNHFRCQVQFYGLSENDEWTQDRAKPVTQIVSAEAWGRAD

SEQ ID NO: 15 - DNA, 339 bp, Artificial Sequence
  nucleotide sequence of TIHDIILECV specific and HLA-A0201 restricted alpha chain variable domain of TCR
gctcagaaggtaactcaagcgcagactgaaatttctgtggtggagaaggaggatgtgaccttggactgtgtgtatgaaacccgtgatactacttattacttattctggtacaagcaaccaccaagtggagaattggttttccttattcgtcggaactcttttgatgagcaaaatgaaataagtggtcggtattcttggaacttccagaaatccaccagttccttcaacttcaccatcacagcctcacaagtcgtggactcagcagtatacttctgtgctctgagggctggggcaaacaacctcttctttgggactggaacgagactcaccgttattccc

SEQ ID NO: 16 - DNA, 342 bp, Artificial Sequence
  nucleotide sequence of TIHDIILECV specific and HLA-A0201 restricted beta chain variable domain of TCR
aatgctggtgtcactcagaccccaaaattccaggtcctgaagacaggacagagcatgacactgcagtgtgcccaggatatgaaccataactccatgtactggtatcgacaagacccaggcatgggactgaggctgatttattactcagcttctgagggtaccactgacaaaggagaagtccccaatggctacaatgtctccagattaaacaaacgggagttctcgctcaggctggagtcggctgctccctcccagacatctgtgtacttctgtgccagcggaccatgggggagctctggaaacaccatatattttggagagggaagttggctcactgttgta

SEQ ID NO: 17 - protein, 5 aa, Artificial Sequence
  beta CDR1
MNHNS

SEQ ID NO: 18 - protein, 6 aa, Artificial Sequence
  beta CDR2
SASEGT

SEQ ID NO: 19 - protein, 13 aa, Artificial Sequence
  beta CDR3
ASGPWGSSGNTIY

SEQ ID NO: 20 - protein, 7 aa, Artificial Sequence
  CDR1alpha
TRDTTYY

SEQ ID NO: 21 - protein, 8 aa, Artificial Sequence
  CDR2alpha
RNSFDEQN

SEQ ID NO: 22 - protein, 10 aa, Artificial Sequence
  CDR3alpha
ALRAGANNLF

SEQ ID NO: 23 - protein, 10 aa, Artificial Sequence
  CDR3alpha
ALRAGANLPV

SEQ ID NO: 24 - protein, 10 aa, Artificial Sequence
  CDR3alpha
ALRAGANTPI

SEQ ID NO: 25 - protein, 10 aa, Artificial Sequence
  CDR3alpha
ALRAGAWPMK